European Patent Specification EP 3 524 618 B1, published March 8, 2023. Title: GLA DOMAINS AS TARGETING AGENTS. Applicant: GLAdiator Biosciences, Inc BAUZON, Maxine HERMISTON, Terry. Application UNKNOWN. The sequence listing filed with the application follows.

SEQUENCE LISTING (6 sequences)

SEQ ID NO: 1 - protein, 45 aa, Artificial sequence
  Synthetic peptide
  misc_feature (6)..(7): X is gamma-carboxyglutamic acid residue
  misc_feature (14)..(14): X is gamma-carboxyglutamic acid residue
  misc_feature (16)..(16): X is gamma-carboxyglutamic acid residue
  misc_feature (19)..(20): X is gamma-carboxyglutamic acid residue
  misc_feature (25)..(26): X is gamma-carboxyglutamic acid residue
  misc_feature (29)..(29): X is gamma-carboxyglutamic acid residue
  misc_feature (32)..(32): X is gamma-carboxyglutamic acid residue
  misc_feature (36)..(36): X is gamma-carboxyglutamic acid residue
ANSLLXXTKQGNLXRXCIXXLCNKXXARXVFXNDPXTDYFYPKYL

SEQ ID NO: 2 - protein, 46 aa, Artificial sequence
  Synthetic peptide
  misc_feature (7)..(8): X is gamma-carboxyglutamic acid residue
  misc_feature (11)..(11): X is gamma-carboxyglutamic acid residue
  misc_feature (15)..(15): X is gamma-carboxyglutamic acid residue
  misc_feature (17)..(17): X is gamma-carboxyglutamic acid residue
  misc_feature (20)..(21): X is gamma-carboxyglutamic acid residue
  misc_feature (26)..(27): X is gamma-carboxyglutamic acid residue
  misc_feature (30)..(30): X is gamma-carboxyglutamic acid residue
  misc_feature (33)..(33): X is gamma-carboxyglutamic acid residue
  misc_feature (35)..(35): X is gamma-carboxyglutamic acid residue
  misc_feature (40)..(40): X is gamma-carboxyglutamic acid residue
AGSYLLXXLFXGNLXKXCYXXICVYXXARXVFXNXVVTDXFWRRYK

SEQ ID NO: 3 - protein, 45 aa, Artificial sequence
  Synthetic peptide
  misc_feature (6)..(7): X is gamma-carboxyglutamic acid residue
  misc_feature (14)..(14): X is gamma-carboxyglutamic acid residue
  misc_feature (16)..(16): X is gamma-carboxyglutamic acid residue
  misc_feature (19)..(20): X is gamma-carboxyglutamic acid residue
  misc_feature (25)..(26): X is gamma-carboxyglutamic acid residue
  misc_feature (29)..(29): X is gamma-carboxyglutamic acid residue
  misc_feature (32)..(32): X is gamma-carboxyglutamic acid residue
ANTFLXXVRKGNLXRXCVXXTCSYXXAFXALXSSTATDVFWAKYT

SEQ ID NO: 4 - protein, 45 aa, Artificial sequence
  Synthetic peptide
  misc_feature (6)..(7): X is gamma-carboxyglutamic acid residue
  misc_feature (14)..(14): X is gamma-carboxyglutamic acid residue
  misc_feature (16)..(16): X is gamma-carboxyglutamic acid residue
  misc_feature (19)..(20): X is gamma-carboxyglutamic acid residue
  misc_feature (25)..(26): X is gamma-carboxyglutamic acid residue
  misc_feature (29)..(29): X is gamma-carboxyglutamic acid residue
  misc_feature (35)..(35): X is gamma-carboxyglutamic acid residue
ANAFLXXLRPGSLXRXCKXXQCSFXXARXIFKDAXRTKLFWISYS

SEQ ID NO: 5 - protein, 45 aa, Artificial sequence
  Synthetic peptide
  misc_feature (6)..(7): X is gamma-carboxyglutamic acid residue
  misc_feature (14)..(14): X is gamma-carboxyglutamic acid residue
  misc_feature (16)..(16): X is gamma-carboxyglutamic acid residue
  misc_feature (19)..(20): X is gamma-carboxyglutamic acid residue
  misc_feature (25)..(26): X is gamma-carboxyglutamic acid residue
  misc_feature (29)..(29): X is gamma-carboxyglutamic acid residue
  misc_feature (32)..(32): X is gamma-carboxyglutamic acid residue
  misc_feature (35)..(35): X is gamma-carboxyglutamic acid residue
ANAFLXXLRQGSLXRXCKXXQCSFXXARXIFXDAXRTKLFWISYS

SEQ ID NO: 6 - protein, 250 aa, Artificial sequence
  Synthetic peptide
  misc_feature (6)..(7): X is gamma-carboxyglutamic acid residue
  misc_feature (14)..(14): X is gamma-carboxyglutamic acid residue
  misc_feature (16)..(16): X is gamma-carboxyglutamic acid residue
  misc_feature (19)..(20): X is gamma-carboxyglutamic acid residue
  misc_feature (25)..(26): X is gamma-carboxyglutamic acid residue
  misc_feature (29)..(29): X is gamma-carboxyglutamic acid residue
  misc_feature (32)..(32): X is gamma-carboxyglutamic acid residue
  misc_feature (36)..(36): X is gamma-carboxyglutamic acid residue
ANSLLXXTKQGNLXRXCIXXLCNKXXARXVFXNDPXTDYFYPKYLVCLRSFQTGLFTAARQSTNAYPDLRSCVNAIPDQCSPLPCNEDGYMSCKDGKASFTCTCKPGWQGEKCEFDINECKDPSNINGGCSQICDNTPGSYHCSCKNGFVMLSNKKDCKDVDECSLKPSICGTAVCKNIPGDFECECPEGYRYNLKSKSCEDIDECSENMCAQLCVNYPGGYTCYCDGKKGFKLAQDQKSCESRHHHHHH